European Patent Specification EP 4 031 665 B1, published July 10, 2024. Title: COMPOSITIONS AND METHODS FOR TEMPLATE-FREE DOUBLE STRANDED GEOMETRIC ENZYMATIC NUCLEIC ACID SYNTHESIS. Applicant: Camena Bioscience Limited Stemple, Derek Harvey, Steven Mankowska, Sylwia Bell, Neil Fraser, Andrew. The sequence listing filed with the application follows.

SEQUENCE LISTING (256 sequences)

SEQ ID NO: 1 - DNA, 28 bp, Artificial Sequence
  Synthetic Sequence
  misc_feature (16)..(28): n is a, c, g, or t
gccatgctgtccaggnnnnnnnnnnnnn

SEQ ID NO: 2 - DNA, 300 bp, Artificial Sequence
  Synthetic Sequence
cgacgtgtctatcgaatacgttgtctgccaacatctgtcgcaaccaatgtaggccggcaatgttaagctgtcgacgatgcaagtcaataagcgaacgagtgctccgtctctctcaacctcatagtgactaggaacgcgtaatgcatgaacaatgccgtcaaccgtcaggtgattaggcgtgtcgattctccgtccttgtacaagacgtggtagaaccggcaatgttcgactctgtcgaagaacgctgtcagagtcaatcaacatctgctcgtgtagttctgtgcaggtatgacggattcc

SEQ ID NO: 3 - DNA, 10 bp, Artificial Sequence
  Synthetic Sequence
gtgtctatcg

SEQ ID NO: 4 - DNA, 10 bp, Artificial Sequence
  Synthetic Sequence
gctgcacaga

SEQ ID NO: 5 - DNA, 24 bp, Artificial Sequence
  Synthetic Sequence
aatacgttgtctgccaacatctgt

SEQ ID NO: 6 - DNA, 24 bp, Artificial Sequence
  Synthetic Sequence
tagcttatgcaacagacggttgta

SEQ ID NO: 7 - DNA, 20 bp, Artificial Sequence
  Synthetic Sequence
cgcaaccaatgtaggccggc

SEQ ID NO: 8 - DNA, 20 bp, Artificial Sequence
  Synthetic Sequence
gacagcgttggttacatccg

SEQ ID NO: 9 - DNA, 27 bp, Artificial Sequence
  Synthetic Sequence
aatgttaagctgtcgacgatgcaagtc

SEQ ID NO: 10 - DNA, 27 bp, Artificial Sequence
  Synthetic Sequence
gccgttacaattcgacagctgctacgt

SEQ ID NO: 11 - DNA, 22 bp, Artificial Sequence
  Synthetic Sequence
aataagcgaacgagtgctccgt

SEQ ID NO: 12 - DNA, 22 bp, Artificial Sequence
  Synthetic Sequence
tcagttattcgcttgctcacga

SEQ ID NO: 13 - DNA, 27 bp, Artificial Sequence
  Synthetic Sequence
ctctctcaacctcatagtgactaggaa

SEQ ID NO: 14 - DNA, 27 bp, Artificial Sequence
  Synthetic Sequence
ggcagagagagttggagtatcactgat

SEQ ID NO: 15 - DNA, 21 bp, Artificial Sequence
  Synthetic Sequence
cgcgtaatgcatgaacaatgc

SEQ ID NO: 16 - DNA, 21 bp, Artificial Sequence
  Synthetic Sequence
ccttgcgcattacgtacttgt

SEQ ID NO: 17 - DNA, 23 bp, Artificial Sequence
  Synthetic Sequence
cgtcaaccgtcaggtgattaggc

SEQ ID NO: 18 - DNA, 23 bp, Artificial Sequence
  Synthetic Sequence
tacggcagttggcagtccactaa

SEQ ID NO: 19 - DNA, 19 bp, Artificial Sequence
  Synthetic Sequence
gtgtcgattctccgtcctt

SEQ ID NO: 20 - DNA, 19 bp, Artificial Sequence
  Synthetic Sequence
tccgcacagctaagaggca

SEQ ID NO: 21 - DNA, 24 bp, Artificial Sequence
  Synthetic Sequence
gtacaagacgtggtagaaccggca

SEQ ID NO: 22 - DNA, 24 bp, Artificial Sequence
  Synthetic Sequence
ggaacatgttctgcaccatcttgg

SEQ ID NO: 23 - DNA, 22 bp, Artificial Sequence
  Synthetic Sequence
atgttcgactctgtcgaagaac

SEQ ID NO: 24 - DNA, 22 bp, Artificial Sequence
  Synthetic Sequence
ccgttacaagctgagacagctt

SEQ ID NO: 25 - DNA, 19 bp, Artificial Sequence
  Synthetic Sequence
gctgtcagagtcaatcaac

SEQ ID NO: 26 - DNA, 19 bp, Artificial Sequence
  Synthetic Sequence
cttgcgacagtctcagtta

SEQ ID NO: 27 - DNA, 21 bp, Artificial Sequence
  Synthetic Sequence
atctgctcgtgtagttctgtg

SEQ ID NO: 28 - DNA, 21 bp, Artificial Sequence
  Synthetic Sequence
gttgtagacgagcacatcaag

SEQ ID NO: 29 - DNA, 17 bp, Artificial Sequence
  Synthetic Sequence
caggtatgacggattcc

SEQ ID NO: 30 - DNA, 17 bp, Artificial Sequence
  Synthetic Sequence
acacgtccatactgcct

SEQ ID NO: 31 - DNA, 34 bp, Artificial Sequence
  Synthetic Sequence
gtgtctatcgaatacgttgtctgccaacatctgt

SEQ ID NO: 32 - DNA, 34 bp, Artificial Sequence
  Synthetic Sequence
gctgcacagatagcttatgcaacagacggttgta

SEQ ID NO: 33 - DNA, 47 bp, Artificial Sequence
  Synthetic Sequence
cgcaaccaatgtaggccggcaatgttaagctgtcgacgatgcaagtc

SEQ ID NO: 34 - DNA, 47 bp, Artificial Sequence
  Synthetic Sequence
gacagcgttggttacatccggccgttacaattcgacagctgctacgt

SEQ ID NO: 35 - DNA, 49 bp, Artificial Sequence
  Synthetic Sequence
aataagcgaacgagtgctccgtctctctcaacctcatagtgactaggaa

SEQ ID NO: 36 - DNA, 49 bp, Artificial Sequence
  Synthetic Sequence
tcagttattcgcttgctcacgaggcagagagagttggagtatcactgat

SEQ ID NO: 37 - DNA, 44 bp, Artificial Sequence
  Synthetic Sequence
cgcgtaatgcatgaacaatgccgtcaaccgtcaggtgattaggc

SEQ ID NO: 38 - DNA, 44 bp, Artificial Sequence
  Synthetic Sequence
ccttgcgcattacgtacttgttacggcagttggcagtccactaa

SEQ ID NO: 39 - DNA, 43 bp, Artificial Sequence
  Synthetic Sequence
gtgtcgattctccgtccttgtacaagacgtggtagaaccggca

SEQ ID NO: 40 - DNA, 43 bp, Artificial Sequence
  Synthetic Sequence
tccgcacagctaagaggcaggaacatgttctgcaccatcttgg

SEQ ID NO: 41 - DNA, 41 bp, Artificial Sequence
  Synthetic Sequence
atgttcgactctgtcgaagaacgctgtcagagtcaatcaac

SEQ ID NO: 42 - DNA, 41 bp, Artificial Sequence
  Synthetic Sequence
ccgttacaagctgagacagcttcttgcgacagtctcagtta

SEQ ID NO: 43 - DNA, 38 bp, Artificial Sequence
  Synthetic Sequence
atctgctcgtgtagttctgtgcaggtatgacggattcc

SEQ ID NO: 44 - DNA, 38 bp, Artificial Sequence
  Synthetic Sequence
gttgtagacgagcacatcaagacacgtccatactgcct

SEQ ID NO: 45 - DNA, 81 bp, Artificial Sequence
  Synthetic Sequence
gtgtctatcgaatacgttgtctgccaacatctgtcgcaaccaatgtaggccggcaatgttaagctgtcgacgatgcaagtc

SEQ ID NO: 46 - DNA, 81 bp, Artificial Sequence
  Synthetic Sequence
gctgcacagatagcttatgcaacagacggttgtagacagcgttggttacatccggccgttacaattcgacagctgctacgt

SEQ ID NO: 47 - DNA, 93 bp, Artificial Sequence
  Synthetic Sequence
aataagcgaacgagtgctccgtctctctcaacctcatagtgactaggaacgcgtaatgcatgaacaatgccgtcaaccgtcaggtgattaggc

SEQ ID NO: 48 - DNA, 93 bp, Artificial Sequence
  Synthetic Sequence
tcagttattcgcttgctcacgaggcagagagagttggagtatcactgatccttgcgcattacgtacttgttacggcagttggcagtccactaa

SEQ ID NO: 49 - DNA, 43 bp, Artificial Sequence; identical to SEQ ID NO: 39
  Synthetic Sequence

SEQ ID NO: 50 - DNA, 43 bp, Artificial Sequence; identical to SEQ ID NO: 40
  Synthetic Sequence

SEQ ID NO: 51 - DNA, 79 bp, Artificial Sequence
  Synthetic Sequence
atgttcgactctgtcgaagaacgctgtcagagtcaatcaacatctgctcgtgtagttctgtgcaggtatgacggattcc

SEQ ID NO: 52 - DNA, 79 bp, Artificial Sequence
  Synthetic Sequence
ccgttacaagctgagacagcttcttgcgacagtctcagttagttgtagacgagcacatcaagacacgtccatactgcct

SEQ ID NO: 53 - DNA, 81 bp, Artificial Sequence; identical to SEQ ID NO: 45
  Synthetic Sequence

SEQ ID NO: 54 - DNA, 85 bp, Artificial Sequence
  Synthetic Sequence
gctgcacagatagcttatgcaacagacggttgtagacagcgttggttacatccggccgttacaattcgacagctgctacgttcag

SEQ ID NO: 55 - DNA, 59 bp, Artificial Sequence
  Synthetic Sequence
gtgtcgattctccgtccttgtacaagacgtggtagaaccggcaatgttcgactctgtcg

SEQ ID NO: 56 - DNA, 63 bp, Artificial Sequence
  Synthetic Sequence
tccgcacagctaagaggcaggaacatgttctgcaccatcttggccgttacaagctgagacagc

SEQ ID NO: 57 - DNA, 35 bp, Artificial Sequence
  Synthetic Sequence
tggacgagacccgccgttcaagacggcgggtctcg

SEQ ID NO: 58 - DNA, 35 bp, Artificial Sequence
  Synthetic Sequence
ctcctgagacccgccgttcaagacggcgggtctca

SEQ ID NO: 59 - DNA, 20 bp, Artificial Sequence
  Synthetic Sequence
tccataagatgcctccacgt

SEQ ID NO: 60 - DNA, 20 bp, Artificial Sequence
  Synthetic Sequence
ggagacgtggaggcatctta

SEQ ID NO: 61 - DNA, 45 bp, Artificial Sequence
  Synthetic Sequence
accctcgtgaccaccttgacctacggcgtgcagtgcttcgcccgc

SEQ ID NO: 62 - DNA, 45 bp, Artificial Sequence
  Synthetic Sequence
tgggagcactggtggaactggatgccgcacgtcacgaagcgggcg

SEQ ID NO: 63 - protein, 15 aa, Artificial Sequence
  Synthetic Sequence
TLVTTLTYGVQCFAR

SEQ ID NO: 64 - DNA, 45 bp, Artificial Sequence
  Synthetic Sequence
cccgacaaccactacctgagcacccagtccgccctgagcaaagac

SEQ ID NO: 65 - DNA, 45 bp, Artificial Sequence
  Synthetic Sequence
gggctgttggtgatggactcgtgggtcaggcgggactgctttctg

SEQ ID NO: 66 - protein, 15 aa, Artificial Sequence
  Synthetic Sequence
PDNHYLSTQSALSKD

SEQ ID NO: 67 - DNA, 21 bp, Artificial Sequence
  Synthetic Sequence
ggcgtgcagtgcttcgcccgc

SEQ ID NO: 68 - DNA, 17 bp, Artificial Sequence
  Synthetic Sequence
acgtcacgaagcgggcg

SEQ ID NO: 69 - DNA, 45 bp, Artificial Sequence; identical to SEQ ID NO: 64
  Synthetic Sequence

SEQ ID NO: 70 - DNA, 45 bp, Artificial Sequence; identical to SEQ ID NO: 65
  Synthetic Sequence

SEQ ID NO: 71 - DNA, 24 bp, Artificial Sequence
  Synthetic Sequence
accctcgtgaccaccttgacctgg

SEQ ID NO: 72 - DNA, 28 bp, Artificial Sequence
  Synthetic Sequence
tgggagcactggtggaactggaccccgc

SEQ ID NO: 73 - DNA, 28 bp, Artificial Sequence
  Synthetic Sequence
gagctaccagtccgccctgagcaaagac

SEQ ID NO: 74 - DNA, 24 bp, Artificial Sequence
  Synthetic Sequence
atggtcaggcgggactgctttctg

SEQ ID NO: 75 - DNA, 45 bp, Artificial Sequence
  Synthetic Sequence
accctcgtgaccaccttgacctggggcgtgcagtgcttcgcccgc

SEQ ID NO: 76 - DNA, 45 bp, Artificial Sequence
  Synthetic Sequence
tgggagcactggtggaactggaccccgcacgtcacgaagcgggcg

SEQ ID NO: 77 - DNA, 45 bp, Artificial Sequence
  Synthetic Sequence
cccgacaaccactacctgagctaccagtccgccctgagcaaagac

SEQ ID NO: 78 - DNA, 45 bp, Artificial Sequence
  Synthetic Sequence
gggctgttggtgatggactcgatggtcaggcgggactgctttctg

SEQ ID NO: 79 - protein, 15 aa, Artificial Sequence
  Synthetic Sequence
TLVTTLTWGVQCFAR

SEQ ID NO: 80 - protein, 15 aa, Artificial Sequence
  Synthetic Sequence
PDNHYLSYQSALSKD

SEQ ID NO: 81 - DNA, 45 bp, Artificial Sequence
  Synthetic Sequence
  misc_feature (22)..(23): n is a, c, g, or t
accctcgtgaccaccttgaccnncggcgtgcagtgcttcgcccgc

SEQ ID NO: 82 - DNA, 45 bp, Artificial Sequence
  Synthetic Sequence
  misc_feature (22)..(23): n is a, c, g, or t
tgggagcactggtggaactggnngccgcacgtcacgaagcgggcg

SEQ ID NO: 83 - protein, 15 aa, Artificial Sequence
  Synthetic Sequence
  misc_feature (8)..(8): Xaa can be any naturally occurring amino acid
TLVTTLTXGVQCFAR

SEQ ID NO: 84 - DNA, 45 bp, Artificial Sequence
  Synthetic Sequence
  misc_feature (22)..(23): n is a, c, g, or t
cccgacaaccactacctgagcnnccagtccgccctgagcaaagac

SEQ ID NO: 85 - DNA, 45 bp, Artificial Sequence
  Synthetic Sequence
  misc_feature (22)..(23): n is a, c, g, or t
gggctgttggtgatggactcgnnggtcaggcgggactgctttctg

SEQ ID NO: 86 - protein, 15 aa, Artificial Sequence
  Synthetic Sequence
  misc_feature (8)..(8): Xaa can be any naturally occurring amino acid
PDNHYLSXQSALSKD

SEQ ID NO: 87 - DNA, 45 bp, Artificial Sequence; identical to SEQ ID NO: 61
  Synthetic Sequence

SEQ ID NO: 88 - DNA, 45 bp, Artificial Sequence; identical to SEQ ID NO: 62
  Synthetic Sequence

SEQ ID NO: 89 - protein, 15 aa, Artificial Sequence
  Synthetic Sequence
TLVTTLTYGVQCFAR

SEQ ID NO: 90 - DNA, 45 bp, Artificial Sequence; identical to SEQ ID NO: 64
  Synthetic Sequence

SEQ ID NO: 91 - DNA, 45 bp, Artificial Sequence; identical to SEQ ID NO: 65
  Synthetic Sequence

SEQ ID NO: 92 - protein, 15 aa, Artificial Sequence
  Synthetic Sequence
PDNHYLSTQSALSKD

SEQ ID NO: 93 - DNA, 13 bp, Artificial Sequence
  Synthetic Sequence
cgtgaccaccttg

SEQ ID NO: 94 - DNA, 13 bp, Artificial Sequence
  Synthetic Sequence
cacgtcacgaagc

SEQ ID NO: 95 - DNA, 16 bp, Artificial Sequence
  Synthetic Sequence
  misc_feature (14)..(15): n is a, c, g, or t
cgtgaccaccttgnnc

SEQ ID NO: 96 - DNA, 12 bp, Artificial Sequence
  Synthetic Sequence
  misc_feature (10)..(11): n is a, c, g, or t
tggtggaacnng

SEQ ID NO: 97 - DNA, 19 bp, Artificial Sequence
  Synthetic Sequence
  misc_feature (14)..(15): n is a, c, g, or t
  misc_feature (17)..(18): n is a, c, g, or t
cgtgaccaccttgnncnnc

SEQ ID NO: 98 - DNA, 15 bp, Artificial Sequence
  Synthetic Sequence
  misc_feature (10)..(11): n is a, c, g, or t
  misc_feature (13)..(14): n is a, c, g, or t
tggtggaacnngnng

SEQ ID NO: 99 - DNA, 22 bp, Artificial Sequence
  Synthetic Sequence
  misc_feature (14)..(15): n is a, c, g, or t
  misc_feature (17)..(18): n is a, c, g, or t
  misc_feature (20)..(21): n is a, c, g, or t
cgtgaccaccttgnncnncnnc

SEQ ID NO: 100 - DNA, 18 bp, Artificial Sequence
  Synthetic Sequence
  misc_feature (10)..(11): n is a, c, g, or t
  misc_feature (13)..(14): n is a, c, g, or t
  misc_feature (16)..(17): n is a, c, g, or t
tggtggaacnngnngnng

SEQ ID NO: 101 - DNA, 25 bp, Artificial Sequence
  Synthetic Sequence
  misc_feature (14)..(15): n is a, c, g, or t
  misc_feature (17)..(18): n is a, c, g, or t
  misc_feature (20)..(21): n is a, c, g, or t
  misc_feature (23)..(24): n is a, c, g, or t
cgtgaccaccttgnncnncnncnnc

SEQ ID NO: 102 - DNA, 21 bp, Artificial Sequence
  Synthetic Sequence
  misc_feature (10)..(11): n is a, c, g, or t
  misc_feature (13)..(14): n is a, c, g, or t
  misc_feature (16)..(17): n is a, c, g, or t
  misc_feature (19)..(20): n is a, c, g, or t
tggtggaacnngnngnngnng

SEQ ID NO: 103 - DNA, 28 bp, Artificial Sequence
  Synthetic Sequence
  misc_feature (14)..(15): n is a, c, g, or t
  misc_feature (17)..(18): n is a, c, g, or t
  misc_feature (20)..(21): n is a, c, g, or t
  misc_feature (23)..(24): n is a, c, g, or t
  misc_feature (26)..(27): n is a, c, g, or t
cgtgaccaccttgnncnncnncnncnnc

SEQ ID NO: 104 - DNA, 24 bp, Artificial Sequence
  Synthetic Sequence
  misc_feature (10)..(11): n is a, c, g, or t
  misc_feature (13)..(14): n is a, c, g, or t
  misc_feature (16)..(17): n is a, c, g, or t
  misc_feature (19)..(20): n is a, c, g, or t
  misc_feature (22)..(23): n is a, c, g, or t
tggtggaacnngnngnngnngnng

SEQ ID NO: 105 - DNA, 40 bp, Artificial Sequence
  Synthetic Sequence
  misc_feature (14)..(15): n is a, c, g, or t
  misc_feature (17)..(18): n is a, c, g, or t
  misc_feature (20)..(21): n is a, c, g, or t
  misc_feature (23)..(24): n is a, c, g, or t
  misc_feature (26)..(27): n is a, c, g, or t
  misc_feature (29)..(30): n is a, c, g, or t
cgtgaccaccttgnncnncnncnncnncnncgtgcagtgc

SEQ ID NO: 106 - DNA, 40 bp, Artificial Sequence
  Synthetic Sequence
  misc_feature (10)..(11): n is a, c, g, or t
  misc_feature (13)..(14): n is a, c, g, or t
  misc_feature (16)..(17): n is a, c, g, or t
  misc_feature (19)..(20): n is a, c, g, or t
  misc_feature (22)..(23): n is a, c, g, or t
  misc_feature (25)..(26): n is a, c, g, or t
tggtggaacnngnngnngnngnngnngcacgtcacgaagc

SEQ ID NO: 107 - DNA, 13 bp, Artificial Sequence
  Synthetic Sequence
cacgtcacgaagc

SEQ ID NO: 108 - protein, 18 aa, Artificial Sequence
  Synthetic Sequence
  misc_feature (7)..(12): Xaa can be any naturally occurring amino acid
TLVTTLXXXXXXVQCFAR

SEQ ID NO: 109 - DNA, 13 bp, Artificial Sequence
  Synthetic Sequence
caaccactacctg

SEQ ID NO: 110 - DNA, 16 bp, Artificial Sequence
  Synthetic Sequence
  misc_feature (14)..(15): n is a, c, g, or t
caaccactacctgnnc

SEQ ID NO: 111 - DNA, 19 bp, Artificial Sequence
  Synthetic Sequence
  misc_feature (14)..(15): n is a, c, g, or t
  misc_feature (17)..(18): n is a, c, g, or t
caaccactacctgnncnnc

SEQ ID NO: 112 - DNA, 22 bp, Artificial Sequence
  Synthetic Sequence
  misc_feature (14)..(15): n is a, c, g, or t
  misc_feature (17)..(18): n is a, c, g, or t
  misc_feature (20)..(21): n is a, c, g, or t
caaccactacctgnncnncnnc

SEQ ID NO: 113 - DNA, 25 bp, Artificial Sequence
  Synthetic Sequence
  misc_feature (14)..(15): n is a, c, g, or t
  misc_feature (17)..(18): n is a, c, g, or t
  misc_feature (20)..(21): n is a, c, g, or t
  misc_feature (23)..(24): n is a, c, g, or t
caaccactacctgnncnncnncnnc

SEQ ID NO: 114 - DNA, 28 bp, Artificial Sequence
  Synthetic Sequence
  misc_feature (14)..(15): n is a, c, g, or t
  misc_feature (17)..(18): n is a, c, g, or t
  misc_feature (20)..(21): n is a, c, g, or t
  misc_feature (23)..(24): n is a, c, g, or t
  misc_feature (26)..(27): n is a, c, g, or t
caaccactacctgnncnncnncnncnnc

SEQ ID NO: 115 - DNA, 40 bp, Artificial Sequence
  Synthetic Sequence
  misc_feature (14)..(15): n is a, c, g, or t
  misc_feature (17)..(18): n is a, c, g, or t
  misc_feature (20)..(21): n is a, c, g, or t
  misc_feature (23)..(24): n is a, c, g, or t
  misc_feature (26)..(27): n is a, c, g, or t
  misc_feature (29)..(30): n is a, c, g, or t
caaccactacctgnncnncnncnncnncnnctccgccctg

SEQ ID NO: 116 - DNA, 12 bp, Artificial Sequence
  Synthetic Sequence
  misc_feature (10)..(11): n is a, c, g, or t
gtgatggacnng

SEQ ID NO: 117 - DNA, 15 bp, Artificial Sequence
  Synthetic Sequence
  misc_feature (10)..(11): n is a, c, g, or t
  misc_feature (13)..(14): n is a, c, g, or t
gtgatggacnngnng

SEQ ID NO: 118 - DNA, 18 bp, Artificial Sequence
  Synthetic Sequence
  misc_feature (10)..(11): n is a, c, g, or t
  misc_feature (13)..(14): n is a, c, g, or t
  misc_feature (16)..(17): n is a, c, g, or t
gtgatggacnngnngnng

SEQ ID NO: 119 - DNA, 21 bp, Artificial Sequence
  Synthetic Sequence
  misc_feature (10)..(11): n is a, c, g, or t
  misc_feature (13)..(14): n is a, c, g, or t
  misc_feature (16)..(17): n is a, c, g, or t
  misc_feature (19)..(20): n is a, c, g, or t
gtgatggacnngnngnngnng

SEQ ID NO: 120 - DNA, 24 bp, Artificial Sequence
  Synthetic Sequence
  misc_feature (10)..(11): n is a, c, g, or t
  misc_feature (13)..(14): n is a, c, g, or t
  misc_feature (16)..(17): n is a, c, g, or t
  misc_feature (19)..(20): n is a, c, g, or t
  misc_feature (22)..(23): n is a, c, g, or t
gtgatggacnngnngnngnngnng

SEQ ID NO: 121 - DNA, 40 bp, Artificial Sequence
  Synthetic Sequence
  misc_feature (10)..(11): n is a, c, g, or t
  misc_feature (13)..(14): n is a, c, g, or t
  misc_feature (16)..(17): n is a, c, g, or t
  misc_feature (19)..(20): n is a, c, g, or t
  misc_feature (22)..(23): n is a, c, g, or t
  misc_feature (25)..(26): n is a, c, g, or t
gtgatggacnngnngnngnngnngnngaggcgggactgct

SEQ ID NO: 122 - DNA, 13 bp, Artificial Sequence
  Synthetic Sequence
aggcgggactgct

SEQ ID NO: 123 - protein, 18 aa, Artificial Sequence
  Synthetic Sequence
  misc_feature (7)..(12): Xaa can be any naturally occurring amino acid
PDNHYLXXXXXXSALSKD

SEQ ID NO: 124 - DNA, 18 bp, Artificial Sequence
  Synthetic Sequence
accctcgtgaccaccttg

SEQ ID NO: 125 - DNA, 21 bp, Artificial Sequence
  Synthetic Sequence
  misc_feature (19)..(20): n is a, c, g, or t
accctcgtgaccaccttgnnc

SEQ ID NO: 126 - DNA, 24 bp, Artificial Sequence
  Synthetic Sequence
  misc_feature (19)..(20): n is a, c, g, or t
  misc_feature (22)..(23): n is a, c, g, or t
accctcgtgaccaccttgnncnnc

SEQ ID NO: 127 - DNA, 27 bp, Artificial Sequence
  Synthetic Sequence
  misc_feature (19)..(20): n is a, c, g, or t
  misc_feature (22)..(23): n is a, c, g, or t
  misc_feature (25)..(26): n is a, c, g, or t
accctcgtgaccaccttgnncnncnnc

SEQ ID NO: 128 - DNA, 30 bp, Artificial Sequence
  Synthetic Sequence
  misc_feature (19)..(20): n is a, c, g, or t
  misc_feature (22)..(23): n is a, c, g, or t
  misc_feature (25)..(26): n is a, c, g, or t
  misc_feature (28)..(29): n is a, c, g, or t
accctcgtgaccaccttgnncnncnncnnc

SEQ ID NO: 129 - DNA, 33 bp, Artificial Sequence
  Synthetic Sequence
  misc_feature (19)..(20): n is a, c, g, or t
  misc_feature (22)..(23): n is a, c, g, or t
  misc_feature (25)..(26): n is a, c, g, or t
  misc_feature (28)..(29): n is a, c, g, or t
  misc_feature (31)..(32): n is a, c, g, or t
accctcgtgaccaccttgnncnncnncnncnnc

SEQ ID NO: 130 - DNA, 54 bp, Artificial Sequence
  Synthetic Sequence
  misc_feature (19)..(20): n is a, c, g, or t
  misc_feature (22)..(23): n is a, c, g, or t
  misc_feature (25)..(26): n is a, c, g, or t
  misc_feature (28)..(29): n is a, c, g, or t
  misc_feature (31)..(32): n is a, c, g, or t
  misc_feature (34)..(35): n is a, c, g, or t
accctcgtgaccaccttgnncnncnncnncnncnncgtgcagtgcttcgcccgc

SEQ ID NO: 131 - DNA, 18 bp, Artificial Sequence
  Synthetic Sequence
tgggagcactggtggaac

SEQ ID NO: 132 - DNA, 21 bp, Artificial Sequence
  Synthetic Sequence
  misc_feature (19)..(20): n is a, c, g, or t
accctcgtgaccaccttgnng

SEQ ID NO: 133 - DNA, 24 bp, Artificial Sequence
  Synthetic Sequence
  misc_feature (19)..(20): n is a, c, g, or t
  misc_feature (22)..(23): n is a, c, g, or t
accctcgtgaccaccttgnngnng

SEQ ID NO: 134 - DNA, 27 bp, Artificial Sequence
  Synthetic Sequence
  misc_feature (19)..(20): n is a, c, g, or t
  misc_feature (22)..(23): n is a, c, g, or t
  misc_feature (25)..(26): n is a, c, g, or t
accctcgtgaccaccttgnngnngnng

SEQ ID NO: 135 - DNA, 30 bp, Artificial Sequence
  Synthetic Sequence
  misc_feature (19)..(20): n is a, c, g, or t
  misc_feature (22)..(23): n is a, c, g, or t
  misc_feature (25)..(26): n is a, c, g, or t
  misc_feature (28)..(29): n is a, c, g, or t
accctcgtgaccaccttgnngnngnngnng

SEQ ID NO: 136 - DNA, 33 bp, Artificial Sequence
  Synthetic Sequence
  misc_feature (19)..(20): n is a, c, g, or t
  misc_feature (22)..(23): n is a, c, g, or t
  misc_feature (25)..(26): n is a, c, g, or t
  misc_feature (28)..(29): n is a, c, g, or t
  misc_feature (31)..(32): n is a, c, g, or t
accctcgtgaccaccttgnngnngnngnngnng

SEQ ID NO: 137 - DNA, 54 bp, Artificial Sequence
  Synthetic Sequence
  misc_feature (19)..(20): n is a, c, g, or t
  misc_feature (22)..(23): n is a, c, g, or t
  misc_feature (25)..(26): n is a, c, g, or t
  misc_feature (28)..(29): n is a, c, g, or t
  misc_feature (31)..(32): n is a, c, g, or t
  misc_feature (34)..(35): n is a, c, g, or t
accctcgtgaccaccttgnngnngnngnngnngnngcacgtcacgaagcgggcg

SEQ ID NO: 138 - protein, 18 aa, Artificial Sequence
  Synthetic Sequence
  misc_feature (7)..(12): Xaa can be any naturally occurring amino acid
TLVTTLXXXXXXVQCFAR

SEQ ID NO: 139 - DNA, 18 bp, Artificial Sequence
  Synthetic Sequence
cccgacaaccactacctg

SEQ ID NO: 140 - DNA, 21 bp, Artificial Sequence
  Synthetic Sequence
  misc_feature (19)..(20): n is a, c, g, or t
cccgacaaccactacctgnnc

SEQ ID NO: 141 - DNA, 24 bp, Artificial Sequence
  Synthetic Sequence
  misc_feature (19)..(20): n is a, c, g, or t
  misc_feature (22)..(23): n is a, c, g, or t
cccgacaaccactacctgnncnnc

SEQ ID NO: 142 - DNA, 27 bp, Artificial Sequence
  Synthetic Sequence
  misc_feature (19)..(20): n is a, c, g, or t
  misc_feature (22)..(23): n is a, c, g, or t
  misc_feature (25)..(26): n is a, c, g, or t
cccgacaaccactacctgnncnncnnc

SEQ ID NO: 143 - DNA, 30 bp, Artificial Sequence
  Synthetic Sequence
  misc_feature (19)..(20): n is a, c, g, or t
  misc_feature (22)..(23): n is a, c, g, or t
  misc_feature (25)..(26): n is a, c, g, or t
  misc_feature (28)..(29): n is a, c, g, or t
cccgacaaccactacctgnncnncnncnnc

SEQ ID NO: 144 - DNA, 33 bp, Artificial Sequence
  Synthetic Sequence
  misc_feature (19)..(20): n is a, c, g, or t
  misc_feature (22)..(23): n is a, c, g, or t
  misc_feature (25)..(26): n is a, c, g, or t
  misc_feature (28)..(29): n is a, c, g, or t
  misc_feature (31)..(32): n is a, c, g, or t
cccgacaaccactacctgnncnncnncnncnnc

SEQ ID NO: 145 - DNA, 54 bp, Artificial Sequence
  Synthetic Sequence
  misc_feature (19)..(20): n is a, c, g, or t
  misc_feature (22)..(23): n is a, c, g, or t
  misc_feature (25)..(26): n is a, c, g, or t
  misc_feature (28)..(29): n is a, c, g, or t
  misc_feature (31)..(32): n is a, c, g, or t
  misc_feature (34)..(35): n is a, c, g, or t
cccgacaaccactacctgnncnncnncnncnncnnctccgccctgagcaaagac

SEQ ID NO: 146 - DNA, 18 bp, Artificial Sequence
  Synthetic Sequence
gggctgttggtgatggac

SEQ ID NO: 147 - DNA, 21 bp, Artificial Sequence
  Synthetic Sequence
  misc_feature (19)..(20): n is a, c, g, or t
gggctgttggtgatggacnng

SEQ ID NO: 148 - DNA, 24 bp, Artificial Sequence
  Synthetic Sequence
  misc_feature (19)..(20): n is a, c, g, or t
  misc_feature (22)..(23): n is a, c, g, or t
gggctgttggtgatggacnngnng

SEQ ID NO: 149 - DNA, 27 bp, Artificial Sequence
  Synthetic Sequence
  misc_feature (19)..(20): n is a, c, g, or t
  misc_feature (22)..(23): n is a, c, g, or t
  misc_feature (25)..(26): n is a, c, g, or t
gggctgttggtgatggacnngnngnng

SEQ ID NO: 150 - DNA, 30 bp, Artificial Sequence
  Synthetic Sequence
  misc_feature (19)..(20): n is a, c, g, or t
  misc_feature (22)..(23): n is a, c, g, or t
  misc_feature (25)..(26): n is a, c, g, or t
  misc_feature (28)..(29): n is a, c, g, or t
gggctgttggtgatggacnngnngnngnng

SEQ ID NO: 151 - DNA, 33 bp, Artificial Sequence
  Synthetic Sequence
  misc_feature (19)..(20): n is a, c, g, or t
  misc_feature (22)..(23): n is a, c, g, or t
  misc_feature (25)..(26): n is a, c, g, or t
  misc_feature (28)..(29): n is a, c, g, or t
  misc_feature (31)..(32): n is a, c, g, or t
gggctgttggtgatggacnngnngnngnngnng

SEQ ID NO: 152 - DNA, 54 bp, Artificial Sequence
  Synthetic Sequence
  misc_feature (19)..(20): n is a, c, g, or t
  misc_feature (22)..(23): n is a, c, g, or t
  misc_feature (25)..(26): n is a, c, g, or t
  misc_feature (28)..(29): n is a, c, g, or t
  misc_feature (31)..(32): n is a, c, g, or t
  misc_feature (34)..(35): n is a, c, g, or t
gggctgttggtgatggacnngnngnngnngnngnngaggcgggactgctttctg

SEQ ID NO: 153 - protein, 18 aa, Artificial Sequence
  Synthetic Sequence
  misc_feature (7)..(12): Xaa can be any naturally occurring amino acid
PDNHYLXXXXXXSALSKD

SEQ ID NO: 154 - DNA, 19 bp, Artificial Sequence
  Synthetic Sequence
gtcgattttttttttagac

SEQ ID NO: 155 - DNA, 19 bp, Artificial Sequence
  Synthetic Sequence
acacccccccccccaatct

SEQ ID NO: 156 - DNA, 19 bp, Artificial Sequence
  Synthetic Sequence
cacgttttttttttttctc

SEQ ID NO: 157 - DNA, 19 bp, Artificial Sequence
  Synthetic Sequence
tctgccccccccccttaca

SEQ ID NO: 158 - DNA, 19 bp, Artificial Sequence
  Synthetic Sequence
  misc_feature (6)..(8): n is a, c, g, or t
gacctnnngactgaatctg

SEQ ID NO: 159 - DNA, 19 bp, Artificial Sequence
  Synthetic Sequence
  misc_feature (12)..(14): n is a, c, g, or t
tcagccacgatnnnttaga

SEQ ID NO: 160 - DNA, 19 bp, Artificial Sequence
  Synthetic Sequence
  misc_feature (6)..(8): n is a, c, g, or t
gtccannngagagtatgac

SEQ ID NO: 161 - DNA, 19 bp, Artificial Sequence
  Synthetic Sequence
  misc_feature (12)..(14): n is a, c, g, or t
agacggtggaannnaatgt

SEQ ID NO: 162 - DNA, 300 bp, Artificial Sequence
  Synthetic Sequence
acaattaatattgttaattaataaccttattgataagtaataatcgaattatatgttaataaccatacgagtctacaatagtggtattaattgaatctgttaatccaactgcctgtagcggtaacttataccgagttaacagtacagtctcacaggcagtgcgacttctgctgctgctcagtcgtgtgtgactgaggcgtagctcagctccggcgaggacacgcggtgctggcacaaccactcgcctcgtcggccaggtggccgccgcctgcgcggccgacgcggccagcgcacgcggtg

SEQ ID NO: 163 - DNA, 300 bp, Artificial Sequence
  Synthetic Sequence
acttaattattagaattatataatggttattcaattgttattaaccattaattacattaattcgatagcacagtactattcaggttataattctatcacaatatcgttctcggacatggccttagaataaccgagtatagagttcagagtgacaggcacaccgtgtacagctccacgactgtgcagagtgtgtgtcgcgatcgacaggtggcggcacgtgagccgctggacggagatcgtctgcgcacgtccggcacctcgccgcgccgtcggccggccacgcgccgtcgcgaccggcag

SEQ ID NO: 164 - DNA, 300 bp, Artificial Sequence
  Synthetic Sequence
tgttaataataacttaattataatgctaatactattcttaattacgttatatatgttatatacgaatcgtcagtagaattgtggaatattaagatagtgattatccaacagcgtgatgccgaatgtattagcgtcaatacacatgactctcagacgctgtggctctacagcacgtcgtgtgaccagtgtgtcacagccgttggacaccagccggcaccactccggcacctcggactacctgagccgtggtcggccacgaccggccggcgacggcgccgcaggccggctgcggtgccggtg

SEQ ID NO: 165 - DNA, 19 bp, Artificial Sequence
  Synthetic Sequence
aattaataaccttattgat

SEQ ID NO: 166 - DNA, 19 bp, Artificial Sequence
  Synthetic Sequence
gcctgcgcggccgacgcgg

SEQ ID NO: 167 - DNA, 19 bp, Artificial Sequence
  Synthetic Sequence
ttatataatggttattcaa

SEQ ID NO: 168 - DNA, 19 bp, Artificial Sequence
  Synthetic Sequence
ccgtcggccggccacgcgc

SEQ ID NO: 169 - DNA, 19 bp, Artificial Sequence
  Synthetic Sequence
aattaataaccttattgat

SEQ ID NO: 170 - DNA, 19 bp, Artificial Sequence
  Synthetic Sequence
gcctgcgcggccgacgcgg

SEQ ID NO: 171 - DNA, 19 bp, Artificial Sequence
  Synthetic Sequence
aattataatgctaatacta

SEQ ID NO: 172 - DNA, 19 bp, Artificial Sequence
  Synthetic Sequence
gcgacggcgccgcaggccg

SEQ ID NO: 173 - DNA, 300 bp, Artificial Sequence
  Synthetic Sequence
ggaataattgttattcaagtcattagtaatagtaatccacttgtaataattacaccttctatacacagacattaatcatgacctctagctgttaatcttgacatgttactgtaacggcagcttgacttcttgacgataggctaatccgaactgtgatctgaagaggcagtcgtgatgcgacggaccaagaggtattgcggatcgtccacactgagcacgtcaggtcgaccgccgcttccaggcattgcaccggtcgtacggcactggcgcgccgcgcgagcgtacgtggcgctccgcagg

SEQ ID NO: 174 - DNA, 300 bp, Artificial Sequence
  Synthetic Sequence
ggtaattatctatatgttctgttatcttattcttatcgtcaagatattaatactggaagattagactctgatattagaacaggagtagctgtaattctagtcatgtaacacttagccgtcgatctgatcatctcgattcggtatagcctagacagttctgaagtgccacaggacatcggtggctgctacacgaattcggcaagcagcacagacaccacctctcgaggagccgccgatccaccgatacgtccgctcgatgcgcagtggccggcgcgccgtggcaaggagcgcgtgcgcacg

SEQ ID NO: 175 - DNA, 300 bp, Artificial Sequence
  Synthetic Sequence
gcaattaatgttattgttgacattacttattgaatacgactagtaataataagagcttcttaacacacagtaattacatctcgtcaaggtgttaatcttgacaacatactgattggccacgatgacttgttgtccttagcgttatggcatcacagaagacatcacgcagagctctacggtcgcaggttgaccaataggcgaaccagctcagacaccagctcaggtggtggcggcctacgtggcaatgctccgctcgttcggctgacggccgccggccgacggttccagcgcgtggcgtgc

SEQ ID NO: 176 - DNA, 19 bp, Artificial Sequence
  Synthetic Sequence
caagtcattagtaatagta

SEQ ID NO: 177 - DNA, 19 bp, Artificial Sequence
  Synthetic Sequence
gcgcgccgcgcgagcgtac

SEQ ID NO: 178 - DNA, 19 bp, Artificial Sequence
  Synthetic Sequence
gttctgttatcttattctt

SEQ ID NO: 179 - DNA, 19 bp, Artificial Sequence
  Synthetic Sequence
gccggcgcgccgtggcaag

SEQ ID NO: 180 - DNA, 19 bp, Artificial Sequence
  Synthetic Sequence
caagtcattagtaatagta

SEQ ID NO: 181 - DNA, 19 bp, Artificial Sequence
  Synthetic Sequence
gcgcgccgcgcgagcgtac

SEQ ID NO: 182 - DNA, 19 bp, Artificial Sequence
  Synthetic Sequence
gttgacattacttattgaa

SEQ ID NO: 183 - DNA, 19 bp, Artificial Sequence
  Synthetic Sequence
ggccgccggccgacggttc

SEQ ID NO: 184 - DNA, 300 bp, Artificial Sequence
  Synthetic Sequence
aatcattaactattatatgtcgttctcaatcaggatgaatcgttgatgttcatacacatgaagaagataaggcttccgttagagaagttagctccatctaactcagagtgttatccagtactctccacaacgaatggtagcagcctgatgatccgttggacgtaagccttatgctcgtaaggtgagctcagaggcaggatcacgcacacaccacagtggtatgccggctacgactgtctgcaccgactgcgtggacgtgtgctgtgcggcttgtccgacgcaagccactgcctcggtccg

SEQ ID NO: 185 - DNA, 300 bp, Artificial Sequence
  Synthetic Sequence
aagtataatgtataacatatgcaactgcataacgatcattgcttgatctgatgttagatgtagttcataaggcttcgcttagacttgaatggtccttgaatctgtgtgtgaactacagttcactggtcaaggttaccatcgaccgagaacatgccatgtctcgtagacgttacgacgattgcacacctgagaggcagcaactggcagtcaggtctgaggtaacggcgcatcgtgtcagagctccgtgtgcctccacctgacgtctccgccaagacggacgcttcgctgacgcagccacgc

SEQ ID NO: 186 - DNA, 300 bp, Artificial Sequence
  Synthetic Sequence
ttcttataactaattcataacgatgtggataagcaagataggttgttctgaagattgtacttgaactaatcgcaaggcatacacatctatccagcatctaagagagtcactagtactgttgagtgcagatccttagcatcgtgccagttcttgcgaagtgtccttctggttacgacgaatgcagtgcactgtccgtcgtagacggtctgacgagagtcgttaccggccatcctgactctccacggagaccgtcctggacagcagaccgccaagtgcgaccgtacgctgtcggagccagcg

SEQ ID NO: 187 - DNA, 19 bp, Artificial Sequence
  Synthetic Sequence
catatgcaactgcataacg

SEQ ID NO: 188 - DNA, 19 bp, Artificial Sequence
  Synthetic Sequence
cgccaagacggacgcttcg

SEQ ID NO: 189 - DNA, 19 bp, Artificial Sequence
  Synthetic Sequence
cataacgatgtggataagc

SEQ ID NO: 190 - DNA, 19 bp, Artificial Sequence
  Synthetic Sequence
cgccaagtgcgaccgtacg

SEQ ID NO: 191 - DNA, 300 bp, Artificial Sequence
  Synthetic Sequence
ctacttcgttatcactaaggcgaatcagagactagttgttatgcagatcaaccttgtacgtacacttgtgagaacgacaagaccaagcttacagtgtgaaggtactcttggacaactctctggttacggattcagccacaactggacgaactcttctctgcaagtgagtagtggtcaccgtatacggagccgaatgcgtctgtgtaccgcatactctgtactgcgcctcattaacgcaccaggcacgtccggtaatgtcgcgtggagatgttggccgcagaatactgaggccgtccgatt

SEQ ID NO: 192 - DNA, 300 bp, Artificial Sequence
  Synthetic Sequence
gtagtacgaattctcattggccatagagagacaacaagattagcacaacttccaacatcgaacactacagtgaaggtgaactggttggatactgactgatccttgtcaacgagttgtctctcgaatgcgaatctggcagttgaggtccttgtgatgagtcgatgtctgatcaggtctggcttaaccgtcgcgtaacggtctcacatggcctatcacagtagaccggcacataatcgctccagcctggaggccattagtcgcgtgctcatcttggcgccacaatagtcaggccgtgcctta

SEQ ID NO: 193 - DNA, 300 bp, Artificial Sequence
  Synthetic Sequence
gttctagcatatgacatacgcctaacacagtgttctagatatcgagaagtagcaagaagctactcatctcacatgctcttctgctaccaatctcagtgtagcaagacttcgtgtagagagacgatagcgaatgaccgagatctcctggttgtctagtcagcaagtgtgatctcctctccgaataggctgcggttagcgtgacagaaggccttagtctcaagacggcgagttattccgtcctccgtgcaggccaatagtccgctggtgttcaagcggcgagtatactcaggcgcaccgtat

SEQ ID NO: 194 - DNA, 19 bp, Artificial Sequence
  Synthetic Sequence
taaggcgaatcagagacta

SEQ ID NO: 195 - DNA, 19 bp, Artificial Sequence
  Synthetic Sequence
gatgttggccgcagaatac

SEQ ID NO: 196 - DNA, 19 bp, Artificial Sequence
  Synthetic Sequence
attggccatagagagacaa

SEQ ID NO: 197 - DNA, 19 bp, Artificial Sequence
  Synthetic Sequence
catcttggcgccacaatag

SEQ ID NO: 198 - DNA, 19 bp, Artificial Sequence
  Synthetic Sequence
taaggcgaatcagagacta

SEQ ID NO: 199 - DNA, 19 bp, Artificial Sequence
  Synthetic Sequence
gatgttggccgcagaatac

SEQ ID NO: 200 - DNA, 19 bp, Artificial Sequence
  Synthetic Sequence
atacgcctaacacagtgtt

SEQ ID NO: 201 - DNA, 18 bp, Artificial Sequence
  Synthetic Sequence
gttcaagcggcgagtatc

SEQ ID NO: 202 - DNA, 300 bp, Artificial Sequence
  Synthetic Sequence
ggaggagacaatggtaatcctagtctcgcatgttctgtgccaaccaatcatcgcggcgaatgataaccacagctcgttcgatctcttaatccgatggagtccaggctcagactgaagcacaatctgagatggtagcgcttaacgttgttcaatccggagtaccgtgtccacttatccggtgtgctatcaggcaccaacatgatgtcgtggaagaagcggctaagatgctcacactcgatcaagcctctgtctgtgtatcatgtagtgctcgtcttctagactgcaggaatcaccgatagg

SEQ ID NO: 203 - DNA, 300 bp, Artificial Sequence; identical to SEQ ID NO: 2
  Synthetic Sequence

SEQ ID NO: 204 - DNA, 300 bp, Artificial Sequence
  Synthetic Sequence
ccacctgtcataggttatggttgagaggcaagatcactccgatgctaagttggcggcgattgttaacgacacctgcttcgaacacaatatggcaaggtctcgacgctcactctgttcgagttactcactaggttggccattacctactacttaggcgagtaggcacaggagtaatcggcagtgcttacagcctccaacatgttgacgtccttcaacggcgtatctacgtgagagagctagatccgagtctcagagattctactagacgtggtgaacaagagtcgtcctatctccgaatcg

SEQ ID NO: 205 - DNA, 19 bp, Artificial Sequence
  Synthetic Sequence
aatcctagtctcgcatgtt

SEQ ID NO: 206 - DNA, 19 bp, Artificial Sequence
  Synthetic Sequence
gctcgtcttctagactgca

SEQ ID NO: 207 - DNA, 19 bp, Artificial Sequence
  Synthetic Sequence
atacgttgtctgccaacat

SEQ ID NO: 208 - DNA, 19 bp, Artificial Sequence
  Synthetic Sequence
gctcgtgtagttctgtgca

SEQ ID NO: 209 - DNA, 19 bp, Artificial Sequence
  Synthetic Sequence
aatcctagtctcgcatgtt

SEQ ID NO: 210 - DNA, 19 bp, Artificial Sequence
  Synthetic Sequence
gctcgtcttctagactgca

SEQ ID NO: 211 - DNA, 19 bp, Artificial Sequence
  Synthetic Sequence
tatggttgagaggcaagat

SEQ ID NO: 212 - DNA, 19 bp, Artificial Sequence
  Synthetic Sequence
cgtggtgaacaagagtcgt

SEQ ID NO: 213 - DNA, 300 bp, Artificial Sequence
  Synthetic Sequence
  misc_feature (21)..(23): n is a, c, g, or t
  misc_feature (278)..(280): n is a, c, g, or t
tctggtcatagaccagacctnnngactgaatctgtgaatgactggactcaggccgactaggtagacgatatccgtcatgtcataatgagctgccatcttcgcgagataggtataggaccggttcatcagccaaggttacgcagacgtgtccgttagtcacttcagttctgatggatgcctgcgcatgaactgatatgctgttcaagaagtctggcagtccacgtcctggccttgtagctatatactatccggataaccgttgccgatcagccacgatnnnttagaccaggaattgcagag

SEQ ID NO: 214 - DNA, 300 bp, Artificial Sequence
  Synthetic Sequence
  misc_feature (21)..(23): n is a, c, g, or t
  misc_feature (278)..(280): n is a, c, g, or t
tcacgtcttacagcagaccannnctgagaatctctgttacacagcagacaccggcagatcctagacgttatgcgtgaagtgattatctgctcggaacttggcgtcaatccataagcagccgatcatcaccgaacctatgcctgaggtgtccgtaagagtgtagagatgacatcctagccaggcgtagaagtgattaccactagatgatcagtggcagtcgacgaccagcggtacttggttaattcattgccgaattccgttccggttgtccgaccttnnnttacacctggattaggtgtg

SEQ ID NO: 215 - DNA, 300 bp, Artificial Sequence
  Synthetic Sequence
  misc_feature (21)..(23): n is a, c, g, or t
  misc_feature (278)..(280): n is a, c, g, or t
tctcgtgtatgtcgtgtccannngagagtatgacagtaactctgctgagaggcgctgtagcttgtccttaacgctcatgtgataatgaggacggatcatccggacaatcctaatcgtgccgtactacaggcaagcatagcctcagctcacggaatcagtgatgtcaactgttccttccgaccgctagttgacattagcacatcaacaactgtcgcagtggtggtccagcgcatgtacgttaatacttaccggaataggctacggctagacggtggaannnaatgtcctcgttaacctcac

SEQ ID NO: 216 - DNA, 19 bp, Artificial Sequence
  Synthetic Sequence
  misc_feature (6)..(8): n is a, c, g, or t
gacctnnngactgaatctg

SEQ ID NO: 217 - DNA, 19 bp, Artificial Sequence
  Synthetic Sequence
  misc_feature (12)..(14): n is a, c, g, or t
tcagccacgatnnnttaga

SEQ ID NO: 218 - DNA, 19 bp, Artificial Sequence
  Synthetic Sequence
  misc_feature (6)..(8): n is a, c, g, or t
gaccannnctgagaatctc

SEQ ID NO: 219 - DNA, 19 bp, Artificial Sequence
  Synthetic Sequence
  misc_feature (12)..(14): n is a, c, g, or t
tgtccgaccttnnnttaca

SEQ ID NO: 220 - DNA, 19 bp, Artificial Sequence
  Synthetic Sequence
  misc_feature (6)..(8): n is a, c, g, or t
gacctnnngactgaatctg

SEQ ID NO: 221 - DNA, 20 bp, Artificial Sequence
  Synthetic Sequence
  misc_feature (13)..(15): n is a, c, g, or t
tcagccaacgatnnnttaga

SEQ ID NO: 222 - DNA, 19 bp, Artificial Sequence
  Synthetic Sequence
  misc_feature (6)..(8): n is a, c, g, or t
gtccannngagagtatgac

SEQ ID NO: 223 - DNA, 19 bp, Artificial Sequence
  Synthetic Sequence
  misc_feature (12)..(14): n is a, c, g, or t
agacggtggaannnaatgt

SEQ ID NO: 224 - DNA, 300 bp, Artificial Sequence
  Synthetic Sequence
tcacgtcttactcgtgtgctaaaaaaaaaaagagagttagtctggactctggcgcacttcgttgagcaatacgcagaagtcaattacacctggcttgatccgcacaatgcattaggacggcaagaactccgatccttaccgtctcgtcagcgatagtcacaacagatgtgaaggatggctcgccatgttgagataagctgatcatgatgactcgctgaggaggtccacgcgatcttggtaataacatagcgcatatcggttgccgaagaggggggggggcattgtgctccaattgcacac

SEQ ID NO: 225 - DNA, 300 bp, Artificial Sequence
  Synthetic Sequence
tctcctgtaactccacaccaaaaaaaaaaatcactcttagagtcctcacaggcggtgtaggaactcgtaatggcacttcagttaatgagcaggcttctacggcacatagcattacgtgccgatctacaggcatggtatgcgtcaggtctccgtaagtcactagtcatgactagcatcgcacggcaagtactgttatgcagaagtagaactctcgctctcgaggtccaggcgttctaggatatatgttaggccaattgcgatgcggtagtggggggggggcatacagcagctaatcgtgtc

SEQ ID NO: 226 - DNA, 300 bp, Artificial Sequence
  Synthetic Sequence
tcaggtgtatgacctgtgctaaaaaaaaaatgagagttagtgacgactgacggccagttccaagtcgttatgcctgttgagataatcagctgccatctaccgctcaatgctaatcgtccggatcaacaccgatcctatcggtcaggacaggctaacagagttgactacagaaccttcggtggccatgttcagaattcgtgatcaacatcactgccagaccagctcgtgcggttgttggattaatcattcggcaattgcctaccggaagaggggggggggctatgtggacgaattccacac

SEQ ID NO: 227 - DNA, 19 bp, Artificial Sequence
  Synthetic Sequence
gtgctaaaaaaaaaaagag

SEQ ID NO: 228 - DNA, 19 bp, Artificial Sequence
  Synthetic Sequence
agaggggggggggcattgt

SEQ ID NO: 229 - DNA, 19 bp, Artificial Sequence
  Synthetic Sequence
caccaaaaaaaaaaatcac

SEQ ID NO: 230 - DNA, 19 bp, Artificial Sequence
  Synthetic Sequence
agtggggggggggcataca

SEQ ID NO: 231 - DNA, 19 bp, Artificial Sequence
  Synthetic Sequence
gtgctaaaaaaaaaaagag

SEQ ID NO: 232 - DNA, 19 bp, Artificial Sequence
  Synthetic Sequence
agaggggggggggcattgt

SEQ ID NO: 233 - DNA, 19 bp, Artificial Sequence
  Synthetic Sequence
gtgctaaaaaaaaaaagag

SEQ ID NO: 234 - DNA, 19 bp, Artificial Sequence
  Synthetic Sequence
agacggggggggggtatgt

SEQ ID NO: 235 - DNA, 300 bp, Artificial Sequence
  Synthetic Sequence
agacgtgaatcaccagtcgattttttttttagactgttagactccagtctggcggtcaaggatcaccattagcctcttctctaatagtcctccgtagttccggacttacctaatggtcggcatgtactccgtacgtatcggacaggtgtcggttactgtcttcagtagagttgcaagcgacgcctagtacagaatacgagatgttcatctcacggacaggtcctggaccggtagaaggaatatacatacggcattaggcatgccgtacacccccccccccaatctccagcattacctgag

SEQ ID NO: 236 - DNA, 300 bp, Artificial Sequence
  Synthetic Sequence
actgctctaacacgtcacgttttttttttttctcagttagagtcctgtgtgccggtcaaccatctccaattccgacatcagattaagaggtccgttcatggcctgtaacgtataggtccggtacaacacggtaggttagcgagtccacaggcaatgagtcatgtctacagtagctagcgagcgcttgtagacaattggagatcaacaactgtggctgacgaccaccaggccttgaagcttataagaatccgcttaaggcttcgccttctgccccccccccttacaggtgcaattgcagtc

SEQ ID NO: 237 - DNA, 300 bp, Artificial Sequence
  Synthetic Sequence
tctccacttacacgtcaggattttttttttagagtctatctcaggtctgagcggctcttggatcaggaattcgctgaactcataatctcctgcctacttccgctgattcgataaccacggcttgaagagcgaagctaaggctctccacagccatagtgtgaacagaactgaagctagcgtcggcttcaagagttatgctcttgaagttgtctgcgtgtccagcacgtcgcgtagtacgaattatgttaggccattacggtaggcgatgagcccccccccctaacaggaccatatccactg

SEQ ID NO: 238 - DNA, 19 bp, Artificial Sequence
  Synthetic Sequence
gtcgattttttttttagac

SEQ ID NO: 239 - DNA, 19 bp, Artificial Sequence
  Synthetic Sequence
acacccccccccccaatct

SEQ ID NO: 240 - DNA, 19 bp, Artificial Sequence
  Synthetic Sequence
cacgttttttttttttctc

SEQ ID NO: 241 - DNA, 19 bp, Artificial Sequence
  Synthetic Sequence
tctgccccccccccttaca

SEQ ID NO: 242 - DNA, 19 bp, Artificial Sequence
  Synthetic Sequence
gtcgattttttttttagac

SEQ ID NO: 243 - DNA, 19 bp, Artificial Sequence
  Synthetic Sequence
acacccccccccccaatct

SEQ ID NO: 244 - DNA, 19 bp, Artificial Sequence
  Synthetic Sequence
caggattttttttttagag

SEQ ID NO: 245 - DNA, 19 bp, Artificial Sequence
  Synthetic Sequence
tgagcccccccccctaaca

SEQ ID NO: 246 - DNA, 300 bp, Artificial Sequence
  Synthetic Sequence
atgcatggctactcggcatctcttcatgagaagcacatggcgattatagccggtaaggtgtcacttgcacgtaaccgtgtgacacacctcttaggaagtctatgacggcgatagccggcatgtatctatcgacacgttgtgtgacacacctcttaggaagtcaactgcgtacataggactacaggctacgtggttacgcacgacatcctatgctggcgagtgttaagcactactgcttgtgtgacacacctcttaggaagtccgaacctacgaaccatgtggtcctatagtgcgttcaag

SEQ ID NO: 247 - DNA, 300 bp, Artificial Sequence
  Synthetic Sequence
accgacgagttacttggcatgattcgaacgaaccgcagtattagacgaggttacgtgacgtctcatctggttccacatgcgtagcctacgtcgtaagcataccagattgtatgcgcttaacgaggtcgccatcctgatatgcgtagcctacgtcgtaagcatatacgaatcgtcgcgtactggtcgtgctccttcaatctattggcaggtccatgagctagataagtcaccaggagcaatgcgtagcctacgtcgtaagcatgtattcgtagcacctaacgtagtgcgaggctaatccag

SEQ ID NO: 248 - DNA, 300 bp, Artificial Sequence
  Synthetic Sequence
tggacagcaagtccagatggataggtccgatctggaggttatccaccatccggattatctaacgcttcttgcagacgcagatctagccaatgatcttggcgcgcaaggtacttgccaattctagttgcacctgagacagcagatctagccaatgatcttggcggaataactgtcctacctcagcgattggcgcgttggttgacaacagaatcttgacgttcacgccagagtgcttacagcagatctagccaatgatcttggcgttgtgctctcaaggctgctactaagatatcggacacg

SEQ ID NO: 249 - DNA, 19 bp, Artificial Sequence
  Synthetic Sequence
gcatctcttcatgagaagc

SEQ ID NO: 250 - DNA, 19 bp, Artificial Sequence
  Synthetic Sequence
cctacgaaccatgtggtcc

SEQ ID NO: 251 - DNA, 19 bp, Artificial Sequence
  Synthetic Sequence
ggcatgattcgaacgaacc

SEQ ID NO: 252 - DNA, 19 bp, Artificial Sequence
  Synthetic Sequence
tcgtagcacctaacgtagt

SEQ ID NO: 253 - DNA, 19 bp, Artificial Sequence
  Synthetic Sequence
gcatctcttcatgagaagc

SEQ ID NO: 254 - DNA, 19 bp, Artificial Sequence
  Synthetic Sequence
cctacgaaccatgtggtcc

SEQ ID NO: 255 - DNA, 19 bp, Artificial Sequence
  Synthetic Sequence
gatggataggtccgatctg

SEQ ID NO: 256 - DNA, 19 bp, Artificial Sequence
  Synthetic Sequence
tgctctcaaggctgctact